European Patent Application EP 4 574 209 A2, published June 25, 2025. Title: METHODS AND TREATMENTS FOR ACNE SCARRING. Applicant: Allergan Pharmaceuticals International Limited. The sequence listing filed with the application follows.

SEQUENCE LISTING (15 sequences)

SEQ ID NO: 1 - protein, 698 aa, synthetic construct
  REGION 1..698: note = SHELdelta26A
GGVPGAIPGGVPGGVFYPGAGLGALGGGALGPGGKPLKPVPGGLAGAGLGAGLGAFPAVTFPGALVPGGVADAAAAYKAAKAGAGLGGVPGVGGLGVSAGAVVPQPGAGVKPGKVPGVGLPGVYPGGVLPGARFPGVGVLPGVPTGAGVKPKAPGVGGAFAGIPGVGPFGGPQPGVPLGYPIKAPKLPGGYGLPYTTGKLPYGYGPGGVAGAAGKAGYPTGTGVGPQAAAAAAAKAAAKFGAGAAGVLPGVGGAGVPGVPGAIPGIGGIAGVGTPAAAAAAAAAAKAAKYGAAAGLVPGGPGFGPGVVGVPGAGVPGVGVPGAGIPVVPGAGIPGAAVPGVVSPEAAAKAAAKAAKYGARPGVGVGGIPTYGVGAGGFPGFGVGVGGIPGVAGVPSVGGVPGVGGVPGVGISPEAQAAAAAKAAKYGVGTPAAAAAKAAAKAAQFGLVPGVGVAPGVGVAPGVGVAPGVGLAPGVGVAPGVGVAPGVGVAPGIGPGGVAAAAKSAAKVAAKAQLRAAAGLGAGIPGLGVGVGVPGLGVGAGVPGLGVGAGVPGFGAVPGALAAAKAAKYGAAVPGVLGGLGALGGVGIPGGVVGAGPAAAAAAAKAAAKAAQFGLVGAAGLGGLGVGGLGVPGVGGLGGIPPAAAAKAAKYGAAGLGGVLGGAGQFPLGGVAARPGFGLSPIFPGGACLGKACGRKRK

SEQ ID NO: 2 - protein, 733 aa, synthetic construct
  REGION 1..733: note = SHEL isoform
SMGGVPGAIPGGVPGGVFYPGAGLGALGGGALGPGGKPLKPVPGGLAGAGLGAGLGAFPAVTFPGALVPGGVADAAAAYKAAKAGAGLGGVPGVGGLGVSAGAVVPQPGAGVKPGKVPGVGLPGVYPGGVLPGARFPGVGVLPGVPTGAGVKPKAPGVGGAFAGIPGVGPFGGPQPGVPLGYPIKAPKLPGGYGLPYTTGKLPYGYGPGGVAGAAGKAGYPTGTGVGPQAAAAAAAKAAAKFGAGAAGVLPGVGGAGVPGVPGAIPGIGGIAGVGTPAAAAAAAAAAKAAKYGAAAGLVPGGPGFGPGVVGVPGAGVPGVGVPGAGIPVVPGAGIPGAAVPGVVSPEAAAKAAAKAAKYGARPGVGVGGIPTYGVGAGGFPGFGVGVGGIPGVAGVPSVGGVPGVGGVPGVGISPEAQAAAAAKAAKYGVGTPAAAAAKAAAKAAQFGLVPGVGVAPGVGVAPGVGVAPGVGLAPGVGVAPGVGVAPGVGVAPGIGPGGVAAAAKSAAKVAAKAQLRAAAGLGAGIPGLGVGVGVPGLGVGAGVPGLGVGAGVPGFGAGADEGVRRSLSPELREGDPSSSQHLPSTPSSPRVPGALAAAKAAKYGAAVPGVLGGLGALGGVGIPGGVVGAGPAAAAAAAKAAAKAAQFGLVGAAGLGGLGVGGLGVPGVGGLGGIPPAAAAKAAKYGAAGLGGVLGGAGQFPLGGVAARPGFGLSPIFPGGACLGKACGRKRK

SEQ ID NO: 3 - protein, 698 aa, synthetic construct; identical to SEQ ID NO: 1
  REGION 1..698: note = SHELdelta26A isoform

SEQ ID NO: 4 - protein, 660 aa, synthetic construct
  REGION 1..660: note = SHELdeltamod isoform
GGVPGAVPGGVPGGVFYPGAGFGAVPGGVADAAAAYKAAKAGAGLGGVPGVGGLGVSAGAVVPQPGAGVKPGKVPGVGLPGVYPGFGAVPGARFPGVGVLPGVPTGAGVKPKAPGVGGAFAGIPGVGPFGGPQPGVPLGYPIKAPKLPGGYGLPYTTGKLPYGYGPGGVAGAAGKAGYPTGTGVGPQAAAAAAAKAAAKFGAGAAGFGAVPGVGGAGVPGVPGAIPGIGGIAGVGTPAAAAAAAAAAKAAKYGAAAGLVPGGPGFGPGVVGVPGFGAVPGVGVPGAGIPVVPGAGIPGAAGFGAVSPEAAAKAAAKAAKYGARPGVGVGGIPTYGVGAGGFPGFGVGVGGIPGVAGVPSVGGVPGVGGVPGVGISPEAQAAAAAKAAKYGVGTPAAAAAKAAAKAAQFGLVPGVGVAPGVGVAPGVGVAPGVGLAPGVGVAPGVGVAPGVGVAPGIGPGGVAAAAKSAAKVAAKAQLRAAAGLGAGIPGLGVGVGVPGLGVGAGVPGLGVGAGVPGFGAVPGALAAAKAAKYGAVPGVLGGLGALGGVGIPGGVVGAGPAAAAAAAKAAAKAAQFGLVGAAGLGGLGVGGLGVPGVGGLGGIPPAAAAKAAKYGAAGLGGVLGGAGQFPLGGVAARPGFGLSPIFPGGACLGKACGRKRK

SEQ ID NO: 5 - protein, 732 aa, synthetic construct
  REGION 1..732: note = Synthetic Sequence
SMGGVPGAIPGGVPGGVFYPGAGLGALGGGALGPGGKPLKPVPGGLAGAGLGAGLGAFPAVTFPGALVPGGVADAAAAYKAAKAGAGLGGVPGVGGLGVSAGAVVPQPGAGVKPGKVPGVGLPGVYPGGVLPGARFPGVGVLPGVPTGAGVKPKAPGVGGAFAGIPGVGPFGGPQPGVPLGYPIKAPKLPGGYGLPYTTGKLPYGYGPGGVAGAAGKAGYPTGTGVGPQAAAAAAAKAAAKFGAGAAGVLPGVGGAGVPGVPGAIPGIGGIAGVGTPAAAAAAAAAAKAAKYGAAAGLVPGGPGFGPGVVGVPGAGVPGVGVPGAGIPVVPGAGIPGAAVPGVVSPEAAAKAAAKAAKYGARPGVGVGGIPTYGVGAGGFPGFGVGVGGIPGVAGVPSVGGVPGVGGVPGVGISPEAQAAAAAKAAKYGVGTPAAAAAKAAAKAAQFGLVPGVGVAPGVGVAPGVGVAPGVGLAPGVGVAPGVGVAPGVGVAPGIGPGGVAAAAKSAAKVAAKAQLRAAAGLGAGIPGLGVGVGVPGLGVGAGVPGLGVGAGVPGFGAGADEGVRRSLSPELREGDPSSSQHLPSTPSSPRVPGALAAAKAAKYGAAVPGVLGGLGALGVGIPGGVVGAGPAAAAAAAKAAAKAAQFGLVGAAGLGGLGVGGLGVPGVGGLGGIPPAAAAKAAKYGAAGLGGVLGGAGQFPLGGVAARPGFGLSPIFPGGACLGKACGRKRK

SEQ ID NO: 6 - protein, 698 aa, synthetic construct; identical to SEQ ID NO: 1
  REGION 1..698: note = Synthetic Sequence

SEQ ID NO: 7 - protein, 660 aa, synthetic construct
  REGION 1..660: note = Synthetic Sequence
MGGVPGAVPGGVPGGVFYPGAGFGAVPGGVADAAAAYKAAKAGAGLGGVPGVGGLGVSAGAVVPQPGAGVKPGKVPGVGLPGVYPGFGAVPGARFPGVGVLPGVPTGAGVKPKAPGVGGAFAGIPGVGPFGGPQPGVPLGYPIKAPKLPGGYGLPYTTGKLPYGYGPGGVAAAGKAGYPTGTGVGPQAAAAAAAKAAAKFGAGAAGFGAVPGVGGAGVPGVPGAIPGIGGIAGVGTPAAAAAAAAAAKAAKYGAAAGLVPGGPGFGPGVVGVPGFGAVPGVGVPGAGIPVVPGAGIPGAAGFGAVSPEAAAKAAAKAAKYGARPGVGVGGIPTYGVGAGFFPGFGVGVGGIPGVAGVPSVGGVPGVGGVPGVGISPEAQAAAAAKAAKYGVGTPAAAAAKAAAKAAQFGLVPGVGVAPGVGVAPGVGVAPGVGLAPGVGVAPGVGVAPGVGVAPGIGPGGVAAAAKSAAKVAAKAQLRAAAGLGAGIPGLGVGVGVPGLGVGAGVPGLGVGAGVPGFGAVPGALAAAKAAKYGAVPGVLGGLGALGGVGIPGGVVGAGPAAAAAAAKAAAKAAQFGLVGAAGLGGLGVGGLGVPGVGGLGGIPPAAAAKAAKYGAAGLGGVLGGAGQFPLGGVAARPGFGLSPIFPGGACLGKACGRKRK

SEQ ID NO: 8 - protein, 147 aa, synthetic construct
  REGION 1..147: note = Synthetic Sequence
SAMGGVPGALAAAKAAKYGAAVPGVLGGLGALGGVGIPGGVVGAGPAAAAAAAKAAAKAAQFGLVGAAGLGGLGVGGLGVPGVGGLGGIPPAAAAKAAKYGAAGLGGVLGGAGQFPLGGVAARPGFGLSPIFPGGACLGKACGRKRK

SEQ ID NO: 9 - protein, 200 aa, synthetic construct
  REGION 1..200: note = Synthetic Sequence
SAMGALVGLGVPGLGVGAGVPGFGAGADEGVRRSLSPELREGDPSSSQHLPSTPSSPRVPGALAAAKAAKYGAAVPGVLGGLGALGGVGIPGGVVGAGPAAAAAAAKAAAKAAQFGLVGAAGLGGLGVGGLGVPGVGGLGGIPPAAAAKAAKYGAAGLGGVLGGAGQFPLGGVAARPGFGLSPIFPGGACLGKACGRKRK

SEQ ID NO: 10 - protein, 60 aa, synthetic construct
  REGION 1..60: note = Synthetic Sequence
GIPPAAAAKAAKYGAAGLGGVLGGAGQFPLGGVAARPGFGLSPIFPGGACLGKACGRKRK

SEQ ID NO: 11 - protein, 47 aa, synthetic construct
  REGION 1..47: note = Synthetic Sequence
GAAGLGGVLGGAGQFPLGGVAARPGFGLSPIFPGGACLGKACGRKRK

SEQ ID NO: 12 - protein, 34 aa, synthetic construct
  REGION 1..34: note = Synthetic Sequence
GADEGVRRSLSPELREGDPSSSQHLPSTPSSPRV

SEQ ID NO: 13 - protein, 34 aa, synthetic construct
  REGION 1..34: note = Synthetic Sequence
GADEGVRRSLSPELREGDPSSSQHLPSTPSSPRF

SEQ ID NO: 14 - protein, 216 aa, synthetic construct
  REGION 1..216: note = Synthetic Sequence
AAAGLGAGIPGLGVGVGVPGLGVGAGVPGLGVGAGVPGFGAGADEGVRRSLSPELREGDPSSSQHLPSTPSSPRVPGALAAAKAAKYGAAVPGVLGGLGALGGVGIPGGVVGAGPAAAAAAAKAAAKAAQFGLVGAAGLGGLGVGGLGVPGVGGLGGIPPAAAAKAAKYGAAGLGGVLGGAGQFPLGGVAARPGFGLSPIFPGGACLGKACGRKRK

SEQ ID NO: 15 - protein, 183 aa, synthetic construct
  REGION 1..183: note = Synthetic Sequence
AAAGLGAGIPGLGVGVGVPGLGVGAGVPGLGVGAGVPGFGAVPGALAAAKAAKYGAAVPGVLGGLGALGGVGIPGGVVGAGPAAAAAAAKAAAKAAQFGLVGAAGLGGLGVGGLGVPGVGGLGGIPPAAAAKAAKYGAAGLGGVLGGAGQFPLGGVAARPGFGLSPIFPGGACLGKACGRKRK